European Patent Specification EP 3 897 844 B1, published November 15, 2023. Title: PHARMACEUTICAL COMBINATION FOR THE TREATMENT OF CANCER. Applicant: Bayer AG. The sequence listing filed with the application follows.

SEQUENCE LISTING (20 sequences)

SEQ ID NO: 1 - protein, 118 aa, Artificial Sequence
  Antibody sequence
QVTLRESGPALVKPTQTLTLTCTFSGFSLSTYGIGVGWIRQPPGKALEWLAHIWWNDNKYYSTSLKTRLTISKDTSKNQVVLTMTNMDPVDTATYYCARISLPYFDYWGQGTTLTVSS

SEQ ID NO: 2 - protein, 7 aa, Artificial Sequence
  Antibody sequence
TYGIGVG

SEQ ID NO: 3 - protein, 16 aa, Artificial Sequence
  Antibody sequence
HIWWNDNKYYSTSLKT

SEQ ID NO: 4 - protein, 8 aa, Artificial Sequence
  Antibody sequence
ISLPYFDY

SEQ ID NO: 5 - protein, 107 aa, Artificial Sequence
  Antibody sequence
DIQLTQSPSFLSASVGDRVTITCKASQNVGTAVAWYQQKPGKAPKLLIYSASNRYTGVPSRFSGSGSGTEFTLTISSLQPEDFATYYCQQYSSYPLTFGGGTKVEIK

SEQ ID NO: 6 - protein, 11 aa, Artificial Sequence
  Antibody sequence
KASQNVGTAVA

SEQ ID NO: 7 - protein, 7 aa, Artificial Sequence
  Antibody sequence
SASNRYT

SEQ ID NO: 8 - protein, 9 aa, Artificial Sequence
  Antibody sequence
QQYSSYPLT

SEQ ID NO: 9 - protein, 443 aa, Artificial Sequence
  Antibody sequence
QVTLRESGPALVKPTQTLTLTCTFSGFSLSTYGIGVGWIRQPPGKALEWLAHIWWNDNKYYSTSLKTRLTISKDTSKNQVVLTMTNMDPVDTATYYCARISLPYFDYWGQGTTLTVSSASTKGPSVFPLAPCSRSTSESTAALGCLVKDYFPEPVTVSWNSGALTSGVHTFPAVLQSSGLYSLSSVVTVPSSNFGTQTYTCNVDHKPSNTKVDKTVERKCCVECPPCPAPPVAGPSVFLFPPKPKDTLMISRTPEVTCVVVDVSHEDPEVQFNWYVDGVEVHNAKTKPREEQFNSTFRVVSVLTVVHQDWLNGKEYKCKVSNKGLPAPIEKTISKTKGQPREPQVYTLPPSREEMTKNQVSLTCLVKGFYPSDIAVEWESNGQPENNYKTTPPMLDSDGSFFLYSKLTVDKSRWQQGNVFSCSVMHEALHNHYTQKSLSLSPG

SEQ ID NO: 10 - protein, 214 aa, Artificial Sequence
  Antibody sequence
DIQLTQSPSFLSASVGDRVTITCKASQNVGTAVAWYQQKPGKAPKLLIYSASNRYTGVPSRFSGSGSGTEFTLTISSLQPEDFATYYCQQYSSYPLTFGGGTKVEIKRTVAAPSVFIFPPSDEQLKSGTASVVCLLNNFYPREAKVQWKVDNALQSGNSQESVTEQDSKDSTYSLSSTLTLSKADYEKHKVYACEVTHQGLSSPVTKSFNRGEC

SEQ ID NO: 11 - protein, 113 aa, Artificial Sequence
  Antibody sequence
EVQLLESGGGLVQPGGSLRLSCAAASGFTFSSYDMSWVRQAPGKGLDWVSTISGGGTYTYYQDSVKGRFTISRDNSKNTLYLQMNSLRAEDTAVYYCASMDYWGQGTTVTVSS

SEQ ID NO: 12 - protein, 5 aa, Artificial Sequence
  Antibody sequence
SYDMS

SEQ ID NO: 13 - protein, 17 aa, Artificial Sequence
  Antibody sequence
TISGGGTYTYYQDSVKG

SEQ ID NO: 14 - protein, 3 aa, Artificial Sequence
  Antibody sequence
MDY

SEQ ID NO: 15 - protein, 107 aa, Artificial Sequence
  Antibody sequence
DIQMTQSPSSLSASVGDRVTITCRASQSIRRYLNWYHQKPGKAPKLLIYGASTLQSGVPSRFSGSGSGTDFTLTISSLQPEDFAVYYCQQSHSAPLTFGGGTKVEIK

SEQ ID NO: 16 - protein, 11 aa, Artificial Sequence
  Antibody sequence
RASQSIRRYLN

SEQ ID NO: 17 - protein, 7 aa, Artificial Sequence
  Antibody sequence
GASTLQS

SEQ ID NO: 18 - protein, 9 aa, Artificial Sequence
  Antibody sequence
QQSHSAPLT

SEQ ID NO: 19 - protein, 440 aa, Artificial Sequence
  Antibody sequence
EVQLLESGGGLVQPGGSLRLSCAAASGFTFSSYDMSWVRQAPGKGLDWVSTISGGGTYTYYQDSVKGRFTISRDNSKNTLYLQMNSLRAEDTAVYYCASMDYWGQGTTVTVSSASTKGPSVFPLAPCSRSTSESTAALGCLVKDYFPEPVTVSWNSGALTSGVHTFPAVLQSSGLYSLSSVVTVPSSSLGTKTYTCNVDHKPSNTKVDKRVESKYGPPCPPCPAPEFLGGPSVFLFPPKPKDTLMISRTPEVTCVVVDVSQEDPEVQFNWYVDGVEVHNAKTKPREEQFNSTYRVVSVLTVLHQDWLNGKEYKCKVSNKGLPSSIEKTISKAKGQPREPQVYTLPPSQEEMTKNQVSLTCLVKGFYPSDIAVEWESNGQPENNYKTTPPVLDSDGSFFLYSRLTVDKSRWQEGNVFSCSVMHEALHNHYTQKSLSLSLGK

SEQ ID NO: 20 - protein, 214 aa, Artificial Sequence
  Antibody sequence
DIQMTQSPSSLSASVGDRVTITCRASQSIRRYLNWYHQKPGKAPKLLIYGASTLQSGVPSRFSGSGSGTDFTLTISSLQPEDFAVYYCQQSHSAPLTFGGGTKVEIKRTVAAPSVFIFPPSDEQLKSGTASVVCLLNNFYPREAKVQWKVDNALQSGNSQESVTEQDSKDSTYSLSSTLTLSKADYEKHKVYACEVTHQGLSSPVTKSFNRGEC